European Patent Specification EP 3 279 217 B1, published November 8, 2023. Title: STREPTOCOCCUS PNEUMONIAE PROTEIN ANTIGEN, AND PREPARATION METHOD AND USE THEREOF. Applicant: CHANGCHUN BCHT BIOTECHNOLOGY CO.; JILIN UNIVERSITY. Application EP16771360.1. The sequence listing filed with the application follows.

SEQUENCE LISTING (16 sequences)

SEQ ID NO: 1 - protein, 290 aa, Streptococcus pneumoniae D39
CASGKKDTTSGQKLKVVATNSIIADITKNIAGDKIDLHSIVPIGQDPHEYEPLPEDVKKTSEADLIFYNGINLETGGNAWFTKLVENAKKTENKDYFAVSDGVDVIYLEGQNEKGKEDPHAWLNLENGIIFAKNIAKQLSAKDPNNKEFYEKNLKEYTDKLDKLDKESKDKFNKIPAEKKLIVTSEGAFKYFSKAYGVPSAYIWEINTEEEGTPEQIKTLVEKLRQTKVPSLFVESSVDDRPMKTVSQDTNIPIYAQIFTDSIAEQGKEGDSYYSMMKYNLDKIAEGLAK

SEQ ID NO: 2 - protein, 288 aa, Streptococcus pneumoniae RX1
EESPVASQSKAEKDYDAAKKDAKNAKKAVEDAQKALDDAKAAQKKYDEDQKKTEEKAALEKAASEEMDKAVAAVQQAYLAYQQATDKAAKDAADKMIDEAKKREEEAKTKFNTVRAMVVPEPEQLAETKKKSEEAKQKAPELTKKLEEAKAKLEEAEKKATEAKQKVDAEEVAPQAKIAELENQVHRLEQELKEIDESESEDYAKEGFRAPLQSKLDAKKAKLSKLEELSDKIDELDAEIAKLEDQLKAAEENNNVEDYFKEGLEKTIAAKKAELEKTEADLKKAVNE

SEQ ID NO: 3 - protein, 75 aa, Streptococcus pneumoniae EF3296
LAKKQTELEKLLDSLDPEGKTQDELDKEAEEAELDKKADELQNKVADLEKEISNLEILLGGADSEDDTAALQNKL

SEQ ID NO: 4 - protein, 378 aa, Artificial sequence
EESPVASQSKAEKDYDAAKKDAKNAKKAVEDAQKALDDAKAAQKKYDEDQKKTEEKAALEKAASEEMDKAVAAVQQAYLAYQQATDKAAKDAADKMIDEAKKREEEAKTKFNTVRAMVVPEPEQLAETKKKSEEAKQKAPELTKKLEEAKAKLEEAEKKATEAKQKVDAEEVAPQAKIAELENQVHRLEQELKEIDESESEDYAKEGFRAPLQSKLDAKKAKLSKLEELSDKIDELDAEIAKLEDQLKAAEENNNVEDYFKEGLEKTIAAKKAELEKTEADLKKAVNEGGGGSGGGGSGGGGSLAKKQTELEKLLDSLDPEGKTQDELDKEAEEAELDKKADELQNKVADLEKEISNLEILLGGADSEDDTAALQNKL

SEQ ID NO: 5 - protein, 683 aa, Artificial sequence
CASGKKDTTSGQKLKVVATNSIIADITKNIAGDKIDLHSIVPIGQDPHEYEPLPEDVKKTSEADLIFYNGINLETGGNAWFTKLVENAKKTENKDYFAVSDGVDVIYLEGQNEKGKEDPHAWLNLENGIIFAKNIAKQLSAKDPNNKEFYEKNLKEYTDKLDKLDKESKDKFNKIPAEKKLIVTSEGAFKYFSKAYGVPSAYIWEINTEEEGTPEQIKTLVEKLRQTKVPSLFVESSVDDRPMKTVSQDTNIPIYAQIFTDSIAEQGKEGDSYYSMMKYNLDKIAEGLAKGGGGSGGGGSGGGGSEESPVASQSKAEKDYDAAKKDAKNAKKAVEDAQKALDDAKAAQKKYDEDQKKTEEKAALEKAASEEMDKAVAAVQQAYLAYQQATDKAAKDAADKMIDEAKKREEEAKTKFNTVRAMVVPEPEQLAETKKKSEEAKQKAPELTKKLEEAKAKLEEAEKKATEAKQKVDAEEVAPQAKIAELENQVHRLEQELKEIDESESEDYAKEGFRAPLQSKLDAKKAKLSKLEELSDKIDELDAEIAKLEDQLKAAEENNNVEDYFKEGLEKTIAAKKAELEKTEADLKKAVNEGGGGSGGGGSGGGGSLAKKQTELEKLLDSLDPEGKTQDELDKEAEEAELDKKADELQNKVADLEKEISNLEILLGGADSEDDTAALQNKL

SEQ ID NO: 6 - DNA, 2049 bp, Artificial sequence
tgcgcgtctggtaaaaaagataccacctctggtcagaaactgaaagttgttgcgaccaactctatcatcgcggatatcaccaaaaacatcgcgggtgataaaatcgatctgcactctatcgttccgatcggtcaggacccgcacgaatacgaaccgctgccggaagatgttaaaaaaacctctgaagcggatctgatcttctacaacggtatcaacctggaaaccggtggtaacgcgtggttcaccaaactggttgaaaacgcgaaaaaaaccgaaaacaaagattacttcgcggtttctgatggtgttgatgttatctacctggaaggtcagaacgaaaaaggtaaagaagatccgcacgcgtggctgaacctggaaaacggtatcatcttcgcgaaaaacatcgcgaaacagctgtctgcgaaagatccgaacaacaaagaattttacgaaaaaaacctgaaagaatacaccgataaactggataaactggataaagaatctaaagataaattcaacaaaatcccggcggaaaaaaaactgatcgttacctctgaaggtgcgttcaaatacttctctaaagcgtacggtgttccgtctgcgtacatctgggaaatcaacaccgaagaagaaggtaccccggaacagatcaaaaccctggttgaaaaactgcgtcagaccaaagttccgtctctgttcgttgaatcttctgttgatgatcgtccgatgaaaaccgtttctcaggataccaacatcccgatctacgcgcagatcttcaccgattctatcgcggaacagggtaaagaaggtgattcttactactctatgatgaaatacaacctggataaaatcgcggaaggtctggcgaaaggtggtggtggttctggtggtggtggttctggtggtggtggttctgaagaatctccggttgcgtctcagtctaaagcggaaaaagattatgatgcggcgaaaaaagatgcgaaaaacgcgaaaaaagcggttgaagatgcgcagaaagcgctggatgatgcgaaagcggcgcagaaaaaatatgatgaagatcagaaaaaaaccgaagaaaaagcggcgctggaaaaagcggcgtctgaagaaatggataaagcggttgcggcggttcagcaggcgtatctggcgtatcagcaggcgaccgataaagcggcgaaagatgcggcggataaaatgatcgatgaagcgaaaaaacgtgaagaagaagcgaaaaccaaattcaacaccgttcgtgcgatggttgttccggaaccggaacagctggcggaaaccaaaaaaaaatctgaagaagcgaaacagaaagcgccggaactgaccaaaaaactggaagaagcgaaagcgaaactggaagaagcggaaaaaaaagcgaccgaagcgaaacagaaagttgatgcggaagaagttgcgccgcaggcgaaaatcgcggaactggaaaaccaggttcaccgtctggaacaggaactgaaagaaatcgatgaatctgaatctgaagattatgcgaaagaaggtttccgtgcgccgctgcagtctaaactggatgcgaaaaaagcgaaactgtctaaactggaagaactgtctgataaaatcgatgaactggatgcggaaatcgcgaaactggaagatcagctgaaagcggcggaagaaaacaacaacgttgaagattatttcaaagaaggtctggaaaaaaccatcgcggcgaaaaaagcggaactggaaaaaaccgaagcggatctgaaaaaagcggttaacgaaggtggtggtggttctggtggtggtggttctggtggtggtggttctctggcgaaaaaacagaccgaactggaaaaactgctggattctctggacccggaaggtaaaacccaggatgaactggataaagaagcggaagaagcggaactggataaaaaagcggatgaactgcagaacaaagttgcggatctggaaaaagaaatctctaacctggaaatcctgctgggtggtgcggattctgaagatgataccgcggcgctgcagaacaaactg

SEQ ID NO: 7 - DNA, 2079 bp, Artificial sequence
catatgcaccaccaccaccaccactgcgcgtctggtaaaaaagataccacctctggtcagaaactgaaagttgttgcgaccaactctatcatcgcggatatcaccaaaaacatcgcgggtgataaaatcgatctgcactctatcgttccgatcggtcaggacccgcacgaatacgaaccgctgccggaagatgttaaaaaaacctctgaagcggatctgatcttctacaacggtatcaacctggaaaccggtggtaacgcgtggttcaccaaactggttgaaaacgcgaaaaaaaccgaaaacaaagattacttcgcggtttctgatggtgttgatgttatctacctggaaggtcagaacgaaaaaggtaaagaagatccgcacgcgtggctgaacctggaaaacggtatcatcttcgcgaaaaacatcgcgaaacagctgtctgcgaaagatccgaacaacaaagaattttacgaaaaaaacctgaaagaatacaccgataaactggataaactggataaagaatctaaagataaattcaacaaaatcccggcggaaaaaaaactgatcgttacctctgaaggtgcgttcaaatacttctctaaagcgtacggtgttccgtctgcgtacatctgggaaatcaacaccgaagaagaaggtaccccggaacagatcaaaaccctggttgaaaaactgcgtcagaccaaagttccgtctctgttcgttgaatcttctgttgatgatcgtccgatgaaaaccgtttctcaggataccaacatcccgatctacgcgcagatcttcaccgattctatcgcggaacagggtaaagaaggtgattcttactactctatgatgaaatacaacctggataaaatcgcggaaggtctggcgaaaggtggtggtggttctggtggtggtggttctggtggtggtggttctgaagaatctccggttgcgtctcagtctaaagcggaaaaagattatgatgcggcgaaaaaagatgcgaaaaacgcgaaaaaagcggttgaagatgcgcagaaagcgctggatgatgcgaaagcggcgcagaaaaaatatgatgaagatcagaaaaaaaccgaagaaaaagcggcgctggaaaaagcggcgtctgaagaaatggataaagcggttgcggcggttcagcaggcgtatctggcgtatcagcaggcgaccgataaagcggcgaaagatgcggcggataaaatgatcgatgaagcgaaaaaacgtgaagaagaagcgaaaaccaaattcaacaccgttcgtgcgatggttgttccggaaccggaacagctggcggaaaccaaaaaaaaatctgaagaagcgaaacagaaagcgccggaactgaccaaaaaactggaagaagcgaaagcgaaactggaagaagcggaaaaaaaagcgaccgaagcgaaacagaaagttgatgcggaagaagttgcgccgcaggcgaaaatcgcggaactggaaaaccaggttcaccgtctggaacaggaactgaaagaaatcgatgaatctgaatctgaagattatgcgaaagaaggtttccgtgcgccgctgcagtctaaactggatgcgaaaaaagcgaaactgtctaaactggaagaactgtctgataaaatcgatgaactggatgcggaaatcgcgaaactggaagatcagctgaaagcggcggaagaaaacaacaacgttgaagattatttcaaagaaggtctggaaaaaaccatcgcggcgaaaaaagcggaactggaaaaaaccgaagcggatctgaaaaaagcggttaacgaaggtggtggtggttctggtggtggtggttctggtggtggtggttctctggcgaaaaaacagaccgaactggaaaaactgctggattctctggacccggaaggtaaaacccaggatgaactggataaagaagcggaagaagcggaactggataaaaaagcggatgaactgcagaacaaagttgcggatctggaaaaagaaatctctaacctggaaatcctgctgggtggtgcggattctgaagatgataccgcggcgctgcagaacaaactgctcgag

SEQ ID NO: 8 - protein, 419 aa, Streptococcus pneumoniae EF5668
EEAPVANQSKAEKDYDAAVKKSEAAKKDYETAKKKAEDAQKKYDEDQKKTEAKAEKERKASEKIAEATKEVQQAYLAYLQASNESQRKEADKKIKEATQRKDEAEAAFATIRTTIVVPEPSELAETKKKAEEATKEAEVAKKKSEEAAKEVEVEKNKILEQDAENEKKIDVLQNKVADLEKGIAPYQNEVAELNKEIARLQSDLKDAEENNVEDYIKEGLEQAITNKKAELATTQQNIDKTQKDLEDAELELEKVLATLDPEGKTQDELDKEAAEAELNEKVEALQNQVAELEEELSKLEDNLKDAETNNVEDYIKEGLEEAIATKKAELEKTQKELDAALNELGPDGDEEETPAPAPQPEKPAEEPENPAPAPKPEKSADQQAEEDYARRSEEEYNRLTQQQPPKAEKPAPAPQPEQP

SEQ ID NO: 9 - DNA, 1257 bp, Artificial sequence
gaagaagcgccggttgcgaaccagtctaaagcggaaaaagattatgatgcggcggttaaaaaatctgaagcggcgaaaaaagattatgaaaccgcgaaaaaaaaagcggaagatgcgcagaaaaaatatgatgaagatcagaaaaaaaccgaagcgaaagcggaaaaagaacgtaaagcgtctgaaaaaatcgcggaagcgaccaaagaagttcagcaggcgtatctggcgtatctgcaggcgtctaacgaatctcagcgtaaagaagcggataaaaaaatcaaagaagcgacccagcgtaaagatgaagcggaagcggcgttcgcgaccatccgtaccaccatcgttgttccggaaccgtctgaactggcggaaaccaaaaaaaaagcggaagaagcgaccaaagaagcggaagttgcgaaaaaaaaatctgaagaagcggcgaaagaagttgaagttgaaaaaaacaaaatcctggaacaggatgcggaaaacgaaaaaaaaatcgatgttctgcagaacaaagttgcggatctggaaaaaggtatcgcgccgtatcagaacgaagttgcggaactgaacaaagaaatcgcgcgtctgcagtctgatctgaaagatgcggaagaaaacaacgttgaagattatatcaaagaaggtctggaacaggcgatcaccaacaaaaaagcggaactggcgaccacccagcagaacatcgataaaacccagaaagatctggaagatgcggaactggaactggaaaaagttctggcgaccctggacccggaaggtaaaacccaggatgaactggataaagaagcggcggaagcggaactgaacgaaaaagttgaagcgctgcagaaccaggttgcggaactggaagaagaactgtctaaactggaagataacctgaaagatgcggaaaccaacaacgttgaagattatatcaaagaaggtctggaagaagcgatcgcgaccaaaaaagcggaactggaaaaaacccagaaagaactggatgcggcgctgaacgaactgggtccggatggtgatgaagaagaaaccccggcgccggcgccgcagccggaaaaaccggcggaagaaccggaaaacccggcgccggcgccgaaaccggaaaaatctgcggatcagcaggcggaagaagattatgcgcgtcgttctgaagaagaatataaccgtctgacccagcagcagccgccgaaagcggaaaaaccggcgccggcgccgcagccggaacagccg

SEQ ID NO: 10 - DNA, 1269 bp, Artificial sequence
catatggaagaagcgccggttgcgaaccagtctaaagcggaaaaagattatgatgcggcggttaaaaaatctgaagcggcgaaaaaagattatgaaaccgcgaaaaaaaaagcggaagatgcgcagaaaaaatatgatgaagatcagaaaaaaaccgaagcgaaagcggaaaaagaacgtaaagcgtctgaaaaaatcgcggaagcgaccaaagaagttcagcaggcgtatctggcgtatctgcaggcgtctaacgaatctcagcgtaaagaagcggataaaaaaatcaaagaagcgacccagcgtaaagatgaagcggaagcggcgttcgcgaccatccgtaccaccatcgttgttccggaaccgtctgaactggcggaaaccaaaaaaaaagcggaagaagcgaccaaagaagcggaagttgcgaaaaaaaaatctgaagaagcggcgaaagaagttgaagttgaaaaaaacaaaatcctggaacaggatgcggaaaacgaaaaaaaaatcgatgttctgcagaacaaagttgcggatctggaaaaaggtatcgcgccgtatcagaacgaagttgcggaactgaacaaagaaatcgcgcgtctgcagtctgatctgaaagatgcggaagaaaacaacgttgaagattatatcaaagaaggtctggaacaggcgatcaccaacaaaaaagcggaactggcgaccacccagcagaacatcgataaaacccagaaagatctggaagatgcggaactggaactggaaaaagttctggcgaccctggacccggaaggtaaaacccaggatgaactggataaagaagcggcggaagcggaactgaacgaaaaagttgaagcgctgcagaaccaggttgcggaactggaagaagaactgtctaaactggaagataacctgaaagatgcggaaaccaacaacgttgaagattatatcaaagaaggtctggaagaagcgatcgcgaccaaaaaagcggaactggaaaaaacccagaaagaactggatgcggcgctgaacgaactgggtccggatggtgatgaagaagaaaccccggcgccggcgccgcagccggaaaaaccggcggaagaaccggaaaacccggcgccggcgccgaaaccggaaaaatctgcggatcagcaggcggaagaagattatgcgcgtcgttctgaagaagaatataaccgtctgacccagcagcagccgccgaaagcggaaaaaccggcgccggcgccgcagccggaacagccgctcgag

SEQ ID NO: 11 - DNA, 882 bp, Artificial sequence
catatgtgcgcgtctggtaaaaaagataccacctctggtcagaaactgaaagttgttgcgaccaactctatcatcgcggatatcaccaaaaacatcgcgggtgataaaatcgatctgcactctatcgttccgatcggtcaggacccgcacgaatacgaaccgctgccggaagatgttaaaaaaacctctgaagcggatctgatcttctacaacggtatcaacctggaaaccggtggtaacgcgtggttcaccaaactggttgaaaacgcgaaaaaaaccgaaaacaaagattacttcgcggtttctgatggtgttgatgttatctacctggaaggtcagaacgaaaaaggtaaagaagatccgcacgcgtggctgaacctggaaaacggtatcatcttcgcgaaaaacatcgcgaaacagctgtctgcgaaagatccgaacaacaaagaattttacgaaaaaaacctgaaagaatacaccgataaactggataaactggataaagaatctaaagataaattcaacaaaatcccggcggaaaaaaaactgatcgttacctctgaaggtgcgttcaaatacttctctaaagcgtacggtgttccgtctgcgtacatctgggaaatcaacaccgaagaagaaggtaccccggaacagatcaaaaccctggttgaaaaactgcgtcagaccaaagttccgtctctgttcgttgaatcttctgttgatgatcgtccgatgaaaaccgtttctcaggataccaacatcccgatctacgcgcagatcttcaccgattctatcgcggaacagggtaaagaaggtgattcttactactctatgatgaaatacaacctggataaaatcgcggaaggtctggcgaaactcgag

SEQ ID NO: 12 - DNA, 1146 bp, Artificial sequence
catatggaagaatctccggttgcgtctcagtctaaagcggaaaaagattatgatgcggcgaaaaaagatgcgaaaaacgcgaaaaaagcggttgaagatgcgcagaaagcgctggatgatgcgaaagcggcgcagaaaaaatatgatgaagatcagaaaaaaaccgaagaaaaagcggcgctggaaaaagcggcgtctgaagaaatggataaagcggttgcggcggttcagcaggcgtatctggcgtatcagcaggcgaccgataaagcggcgaaagatgcggcggataaaatgatcgatgaagcgaaaaaacgtgaagaagaagcgaaaaccaaattcaacaccgttcgtgcgatggttgttccggaaccggaacagctggcggaaaccaaaaaaaaatctgaagaagcgaaacagaaagcgccggaactgaccaaaaaactggaagaagcgaaagcgaaactggaagaagcggaaaaaaaagcgaccgaagcgaaacagaaagttgatgcggaagaagttgcgccgcaggcgaaaatcgcggaactggaaaaccaggttcaccgtctggaacaggaactgaaagaaatcgatgaatctgaatctgaagattatgcgaaagaaggtttccgtgcgccgctgcagtctaaactggatgcgaaaaaagcgaaactgtctaaactggaagaactgtctgataaaatcgatgaactggatgcggaaatcgcgaaactggaagatcagctgaaagcggcggaagaaaacaacaacgttgaagattatttcaaagaaggtctggaaaaaaccatcgcggcgaaaaaagcggaactggaaaaaaccgaagcggatctgaaaaaagcggttaacgaaggtggtggtggttctggtggtggtggttctggtggtggtggttctctggcgaaaaaacagaccgaactggaaaaactgctggattctctggacccggaaggtaaaacccaggatgaactggataaagaagcggaagaagcggaactggataaaaaagcggatgaactgcagaacaaagttgcggatctggaaaaagaaatctctaacctggaaatcctgctgggtggtgcggattctgaagatgataccgcggcgctgcagaacaaactgctcgag

SEQ ID NO: 13 - DNA, 28 bp, Artificial sequence
catatgtgcgcgtctggtaaaaaagata

SEQ ID NO: 14 - DNA, 27 bp, Artificial sequence
ctcgagtttcgccagaccttccgcgat

SEQ ID NO: 15 - DNA, 27 bp, Artificial sequence
catatggaagaatctccggttgcgtct

SEQ ID NO: 16 - DNA, 27 bp, Artificial sequence
ctcgagcagtttgttctgcagcgccgc